European Patent Specification EP 3 802 870 B1, published December 10, 2025. Title: AMPLIFICATION METHOD AND PRIMERS FOR USE THEREIN. Applicant: Monoquant Pty Ltd. The sequence listing filed with the application follows.

SEQUENCE LISTING (21 sequences)

SEQ ID NO: 1 - DNA, 30 bp, Artificial Sequence
  AAMJ1b
ctttgctgagcacctgtccccaagtctgaa

SEQ ID NO: 2 - DNA, 23 bp, Artificial Sequence
  AAMJ2
aggccggctgcagaccccagata

SEQ ID NO: 3 - DNA, 26 bp, Artificial Sequence
  AAMJ3c
cccccggacattatctcccagctcca

SEQ ID NO: 4 - DNA, 34 bp, Artificial Sequence
  AAMJ4c
gcttatttccccccaaaaatgcagcaaaaccctt

SEQ ID NO: 5 - DNA, 32 bp, Artificial Sequence
  AAMJ5c
cctccaaaatgcctccaagactctgaccctga

SEQ ID NO: 6 - DNA, 31 bp, Artificial Sequence
  AAMJ6c
aggaaaccccacaggcagtagcagaaaacaa

SEQ ID NO: 7 - DNA, 31 bp, Artificial Sequence
  TCR1.1b
ttccctgtgacggatctgcaaaagaacctga

SEQ ID NO: 8 - DNA, 31 bp, Artificial Sequence
  TCR1.2b
ccctcctagagacccccagccttacctacaa

SEQ ID NO: 9 - DNA, 31 bp, Artificial Sequence
  TCR1.3b
caagttcccagctgtccagccttgacttact

SEQ ID NO: 10 - DNA, 39 bp, Artificial Sequence
  TCR1.4b
ccaggaactccgaccttatgatacactatcccgaaagaa

SEQ ID NO: 11 - DNA, 34 bp, Artificial Sequence
  TCR1.5b
atggccataccaccctgattctgcaacttaccta

SEQ ID NO: 12 - DNA, 28 bp, Artificial Sequence
  TCR1.6b
gagtcaagagtggagcccccatacctgt

SEQ ID NO: 13 - DNA, 27 bp, Artificial Sequence
  TCR2.1b
cacctggagcccccttcttacctagca

SEQ ID NO: 14 - DNA, 21 bp, Artificial Sequence
  TCR2.2b
cggagccccaaccgcctcctt

SEQ ID NO: 15 - DNA, 22 bp, Artificial Sequence
  TCR2.3b
ggagccccgcttaccgagcact

SEQ ID NO: 16 - DNA, 16 bp, Artificial Sequence
  TCR2.4b
ccggcggccccagctt

SEQ ID NO: 17 - DNA, 20 bp, Artificial Sequence
  TCR2.5b
gcgctcaccgagcaccagga

SEQ ID NO: 18 - DNA, 22 bp, Artificial Sequence
  TCR2.5c
ccgcgctcaccgagcaccagga

SEQ ID NO: 19 - DNA, 23 bp, Artificial Sequence
  TCR2.5d
cccgcgctcaccgagcaccagga

SEQ ID NO: 20 - DNA, 25 bp, Artificial Sequence
  TCR2.6b
cgcgaaaactcacccagcacggtca

SEQ ID NO: 21 - DNA, 23 bp, Artificial Sequence
  TCR2.7d
ggaaggtggggagacgcccgaat